European Patent Specification EP 4 367 236 B1, published May 27, 2026. Title: HIGH-THROUGHPUT CELLULAR MOLECULAR FUNCTION ASSAY SYSTEM AND METHOD. Applicant: Heligenics, Inc. Application US. The sequence listing filed with the application follows.

SEQUENCE LISTING (2 sequences)

SEQ ID NO: 1 - DNA, 14 bp, synthetic construct
  source 1..14: mol_type = other DNA
  misc_feature 5..7: note = Repeat at least once.
aattcngcgatcgc

SEQ ID NO: 2 - DNA, 32 bp, synthetic construct
  source 1..32: mol_type = other DNA
agacgtaccaacaaaagacaatgacaaaaagg